European Patent Specification EP 4 384 223 B1, published October 1, 2025. Title: CYTOTOXICITY TARGETING CHIMERAS FOR CCR2-EXPRESSING CELLS. Applicant: GlaxoSmithKline Intelluctual Property Development. Application US. The sequence listing filed with the application follows.

SEQUENCE LISTING (14 sequences)

SEQ ID NO: 1 - protein, 5 aa, synthetic construct
NYWMS

SEQ ID NO: 2 - protein, 17 aa, synthetic construct
DIHGNRGFNYHASWAKG

SEQ ID NO: 3 - protein, 9 aa, synthetic construct
ADDSGSHDI

SEQ ID NO: 4 - protein, 12 aa, synthetic construct
QSSQSVYSAKLS

SEQ ID NO: 5 - protein, 7 aa, synthetic construct
YGSTLAS

SEQ ID NO: 6 - protein, 12 aa, synthetic construct
QGTFYGPDWYFA

SEQ ID NO: 7 - protein, 116 aa, synthetic construct
EVQLVESGGGLVQPGGSLRLSCAASGFTFSNYWMSWVRQAPGKGLEWVGDIHGNRGFNYHASWAKGRFTVSRSKNTLYLQMNSLRAEDTAVYYCAKADDSGSHDIWGQGTLVTVSS

SEQ ID NO: 8 - protein, 111 aa, synthetic construct
DIQMTQSPSSLSASVGDRVTITCQSSQSVYSAKLSWYQQKPGKAPKLLIYYGSTLASGVPSRFSGSGSGTQFTLTISSLQPEDFATYYCQGTFYGPDWYFAFGGGTKVEIK

SEQ ID NO: 9 - protein, 446 aa, synthetic construct
EVQLVESGGGLVQPGGSLRLSCAASGFTFSNYWMSWVRQAPGKGLEWVGDIHGNRGFNYHASWAKGRFTVSRSKNTLYLQMNSLRAEDTAVYYCAKADDSGSHDIWGQGTLVTVSSASTKGPSVFPLAPSSKSTSGGTAALGCLVKDYFPEPVTVSWNSGALTSGVHTFPAVLQSSGLYSLSSVVTVPSSSLGTQTYICNVNHKPSNTKVDKKVEPKSCDKTHTCPPCPAPELLGGPDVFLFPPKPKDTLMISRTPEVTCVVVDVSHEDPEVKFNWYVDGVEVHNAKTKPREEQYNSTYRVVSVLTVLHQDWLNGKEYKCKVSNKALPAPEEKTISKAKGQPREPQVYTLPPSRDELTKNQVSLTCLVKGFYPSDIAVEWESNGQPENNYKTTPPVLDSDGSFFLYSKLTVDKSRWQQGNVFSCSVMHEALHNHYTQKSLSLSPGK

SEQ ID NO: 10 - protein, 218 aa, synthetic construct
DIQMTQSPSSLSASVGDRVTITCQSSQSVYSAKLSWYQQKPGKAPKLLIYYGSTLASGVPSRFSGSGSGTQFTLTISSLQPEDFATYYCQGTFYGPDWYFAFGGGTKVEIKRTVAAPSVFIFPPSDEQLKSGTASVVCLLNNFYPREAKVQWKVDNALQSGNSQESVTEQDSKDSTYSLSSTLTLSKADYEKHKVYACEVTHQGLSSPVTKSFNRGEC

SEQ ID NO: 11 - protein, 446 aa, synthetic construct
QQQLVESGGRLVTPGGSLTLTCTASGFSLNNYWMSWVRQAPGKGLEWIGDIHGNRGFNYHASWAKGRFTVSRTSTTVDLRMTSLTTEDTAIYFCARADDSGSHDIWGPGTLVTVSSASTKGPSVFPLAPSSKSTSGGTAALGCLVKDYFPEPVTVSWNSGALTSGVHTFPAVLQSSGLYSLSSVVTVPSSSLGTQTYICNVNHKPSNTKVDKKVEPKSCDKTHTCPPCPAPELLGGPDVFLFPPKPKDTLMISRTPEVTCVVVDVSHEDPEVKFNWYVDGVEVHNAKTKPREEQYNSTYRVVSVLTVLHQDWLNGKEYKCKVSNKALPAPEEKTISKAKGQPREPQVYTLPPSRDELTKNQVSLTCLVKGFYPSDIAVEWESNGQPENNYKTTPPVLDSDGSFFLYSKLTVDKSRWQQGNVFSCSVMHEALHNHYTQKSLSLSPGK

SEQ ID NO: 12 - protein, 218 aa, synthetic construct
ELDLTQTPSPVSAAVGDTVTINCQSSQSVYSAKLSWYQQKPGQPPKLLIYYGSTLASGVPSRFKGSGSGTQFSLTISDVQCADAATYYCQGTYYGPDWYFAFGGGTEVVVKRTVAAPSVFIFPPSDEQLKSGTASVVCLLNNFYPREAKVQWKVDNALQSGNSQESVTEQDSKDSTYSLSSTLTLSKADYEKHKVYACEVTHQGLSSPVTKSFNRGEC

SEQ ID NO: 13 - protein, 446 aa, synthetic construct
QQQLVESGGRLVTPGGSLTLTCTASGFSLNNYWMSWVRQAPGKGLEWIGDIHGNRGFNYHASWAKGRFTVSRTSTTVDLRMTSLTTEDTAIYFCARADDSGSHDIWGPGTLVTVSSAKTTAPSVYPLAPVCGDTTGSSVTLGCLVKGYFPEPVTLTWNSGSLSSGVHTFPAVLQSDLYTLSSSVTVTSSTWPSQSITCNVAHPASSTKVDKKIEPRGPTIKPCPPCKCPAPNLLGGPSVFIFPPKIKDVLMISLSPMVTCVVVDVSEDDPDVQISWFVNNVEVLTAQTQTHREDYNSTLRVVSALPIQHQDWMSGKEFKCKVNNKALPAPIERTISKPKGSVRAPQVYVLPPPEEEMTKKQVTLTCMVTDFMPEDIYVEWTNNGKTELNYKNTEPVLDSDGSYFMYSKLRVEKKNWVERNSYSCSVVHEGLHNHHTTKSFSRTPGK

SEQ ID NO: 14 - protein, 218 aa, synthetic construct
ELDLTQTPSPVSAAVGDTVTINCQSSQSVYSAKLSWYQQKPGQPPKLLIYYGSTLASGVPSRFKGSGSGTQFSLTISDVQCADAATYYCQGTYYGPDWYFAFGGGTEVVVKRADAAPTVSIFPPSSEQLTSGGASVVCFLNNFYPKDINVKWKIDGSERQNGVLNSWTDQDSKDSTYSMSSTLTLTKDEYERHNSYTCEATHKTSTSPIVKSFNRNEC